European Patent Specification EP 3 390 663 B1, published April 17, 2024. Title: Method for the detection of a sexually transmitted infectious pathogen. Applicant: SelfDiagnostics Deutschland GmbH. The sequence listing filed with the application follows.

SEQUENCE LISTING (28 sequences)

SEQ ID NO: 1 - protein, 38 aa, Hyalophora cecropia
MPKWKVFKKIEKVGRNIRNGIVKAGPAIAVLGEAKALG

SEQ ID NO: 2 - protein, 31 aa, Ascaris suum
SWLSKTAKKLENSAKKRISEGIAIAIQGGPR

SEQ ID NO: 3 - DNA, 20 bp, Chlamydia trachomatis
ctccttggagcattgtctgg

SEQ ID NO: 4 - DNA, 20 bp, Chlamydia trachomatis
cggatgcgatgaacagtttg

SEQ ID NO: 5 - DNA, 20 bp, Chlamydia trachomatis
aatatcatctttgcggttgc

SEQ ID NO: 6 - DNA, 21 bp, Chlamydia trachomatis
tctacaagagtacatcggtca

SEQ ID NO: 7 - DNA, 39 bp, Chlamydia trachomatis
tcgagcaaccgctgtgacgaccttcattatgtcggagtc

SEQ ID NO: 8 - DNA, 39 bp, Chlamydia trachomatis
gcagcttgtagtcctgcttgagtcttcgtaactcgctcc

SEQ ID NO: 9 - DNA, 18 bp, Chlamydia trachomatis
tacaaacgcctagggtgc

SEQ ID NO: 10 - DNA, 18 bp, Chlamydia trachomatis
cgggcgatttgccttaac

SEQ ID NO: 11 - DNA, 22 bp, Neisseria gonorrhoeae
gctctgactccattatcctatg

SEQ ID NO: 12 - DNA, 19 bp, Neisseria gonorrhoeae
gcattcagacgtgcttcta

SEQ ID NO: 13 - DNA, 39 bp, Neisseria gonorrhoeae
ttgccgcctaaggttccgagctatggcattaggattgtc

SEQ ID NO: 14 - DNA, 40 bp, Neisseria gonorrhoeae
tggaacgagccaaggtgttctcttgcatcaactgttccat

SEQ ID NO: 15 - DNA, 19 bp, Neisseria gonorrhoeae
gcggtcattgacgaaatgg

SEQ ID NO: 16 - DNA, 20 bp, Neisseria gonorrhoeae
aatcaagaataccgcctcac

SEQ ID NO: 17 - DNA, 20 bp, Neisseria gonorrhoeae
aatcaagaataccgcctcac

SEQ ID NO: 18 - DNA, 20 bp, Neisseria gonorrhoeae
agttctacgaacacttgctg

SEQ ID NO: 19 - DNA, 37 bp, Neisseria gonorrhoeae
ttggagatgtggcgttcggacgacatcaacaacgacc

SEQ ID NO: 20 - DNA, 36 bp, Neisseria gonorrhoeae
cggaagcaggcgtcatcagttgtttggtcgcaagga

SEQ ID NO: 21 - DNA, 18 bp, Neisseria gonorrhoeae
tgtccaatgcgtcgttga

SEQ ID NO: 22 - DNA, 18 bp, Neisseria gonorrhoeae
cgccatgccgacaattac

SEQ ID NO: 23 - DNA, 18 bp, Neisseria gonorrhoeae
gacgtcaagtcctcatgg

SEQ ID NO: 24 - DNA, 20 bp, Neisseria gonorrhoeae
cggttaccctacctacttct

SEQ ID NO: 25 - DNA, 40 bp, Neisseria gonorrhoeae
ttgtgagattggctccgctctcacacgtcatacaatggtc

SEQ ID NO: 26 - DNA, 40 bp, Neisseria gonorrhoeae
tcgagtgcatgaagtcggaatcgaacgtattcaccgcagt

SEQ ID NO: 27 - DNA, 19 bp, Neisseria gonorrhoeae
gcttggctaccctctgtac

SEQ ID NO: 28 - DNA, 21 bp, Neisseria gonorrhoeae
ctagtaatcgcaggtcagcat